European Patent Specification EP 3 822 345 B1, published October 16, 2024. Title: GENETICALLY ENGINEERED CELL AND APPLICATION THEREOF. Applicant: CARSGEN THERAPEUTICS CO., LTD. SHANGHAI CANCER INSTITUTE. Application EP19803938.0. The sequence listing filed with the application follows.

SEQUENCE LISTING (35 sequences)

SEQ ID NO: 1 - DNA, 741 bp, Artificial Sequence
  Hu8E5-2I scFV Nucleic acid sequence
caggtgcagctgcaggagagcggccccggcctgatcaagcccagccagaccctgagcctgacctgcaccgtgagcggcggcagcatcagcagcggctacaactggcactggatccggcagccccccggcaagggcctggagtggatcggctacatccactacaccggcagcaccaactacaaccccgccctgcggagccgggtgaccatcagcgtggacaccagcaagaaccagttcagcctgaagctgagcagcgtgaccgccgccgacaccgccatctactactgcgcccggatctacaacggcaacagcttcccctactggggccagggcaccaccgtgaccgtgagcagcggtggaggcggttcaggcggaggtggttctggcggtggcggatcggacatcgtgatgacccagagccccgacagcctggccgtgagcctgggcgagcgggccaccatcaactgcaagagcagccagagcctgttcaacagcggcaaccagaagaactacctgacctggtaccagcagaagcccggccagccccccaagctgctgatctactgggccagcacccgggagagcggcgtgcccgaccggttcagcggcagcggcagcggcaccgacttcaccctgaccatcagcagcctgcaggccgaggacgtggccgtgtactactgccagaacgcctacagcttcccctacaccttcggcggcggcaccaagctggagatcaagcgg

SEQ ID NO: 2 - protein, 247 aa, Artificial Sequence
  Hu8E5-2I scFV amino acid sequence
QVQLQESGPGLIKPSQTLSLTCTVSGGSISSGYNWHWIRQPPGKGLEWIGYIHYTGSTNYNPALRSRVTISVDTSKNQFSLKLSSVTAADTAIYYCARIYNGNSFPYWGQGTTVTVSSGGGGSGGGGSGGGGSDIVMTQSPDSLAVSLGERATINCKSSQSLFNSGNQKNYLTWYQQKPGQPPKLLIYWASTRESGVPDRFSGSGSGTDFTLTISSLQAEDVAVYYCQNAYSFPYTFGGGTKLEIKR

SEQ ID NO: 3 - DNA, 81 bp, Artificial Sequence
  mouse CD8 alpha signal peptide nucleic acid sequence
atggcctcaccgttgacccgctttctgtcgctgaacctgctgctgctgggtgagtcgattatcctggggagtggagaagct

SEQ ID NO: 4 - protein, 27 aa, Artificial Sequence
  mouse CD8 alpha signal peptide nucleic acid sequence
MASPLTRFLSLNLLLLGESIILGSGEA

SEQ ID NO: 5 - DNA, 216 bp, Artificial Sequence
  mouse CD8 hinge region+transmembrane domain nucleic acid sequence
actactaccaagccagtgctgcgaactccctcacctgtgcaccctaccgggacatctcagccccagagaccagaagattgtcggccccgtggctcagtgaaggggaccggattggacttcgcctgtgatatttacatctgggcacccttggccggaatctgcgtggcccttctgctgtccttgatcatcactctcatctgctaccacaggagccga

SEQ ID NO: 6 - protein, 72 aa, Artificial Sequence
  mouse CD8 hinge region+transmembrane domain nucleic acid sequence
TTTKPVLRTPSPVHPTGTSQPQRPEDCRPRGSVKGTGLDFACDIYIWAPLAGICVALLLSLIITLICYHRSR

SEQ ID NO: 7 - DNA, 123 bp, Artificial Sequence
  mouse CD28 intracellular domain nucleic acid sequence
aatagtagaaggaacagactccttcaaagtgactacatgaacatgactccccggaggcctgggctcactcgaaagccttaccagccctacgcccctgccagagactttgcagcgtaccgcccc

SEQ ID NO: 8 - protein, 41 aa, Artificial Sequence
  mouse CD28 intracellular domain nucleic acid sequence
NSRRNRLLQSDYMNMTPRRPGLTRKPYQPYAPARDFAAYRP

SEQ ID NO: 9 - DNA, 321 bp, Artificial Sequence
  intracellular segment CD3xi nucleic acid sequence of mouse CD3
agcaggagtgcagagactgctgccaacctgcaggaccccaaccagctctacaatgagctcaatctagggcgaagagaggaatatgacgtcttggagaagaagcgggctcgggatccagagatgggaggcaaacagcagaggaggaggaacccccaggaaggcgtatacaatgcactgcagaaagacaagatggcagaagcctacagtgagatcggcacaaaaggcgagaggcggagaggcaaggggcacgatggcctttaccagggtctcagcactgccaccaaggacacctatgatgccctgcatatgcagaccctggcc

SEQ ID NO: 10 - protein, 107 aa, Artificial Sequence
  intracellular segment CD3xi amino acid sequence of mouse CD3
SRSAETAANLQDPNQLYNELNLGRREEYDVLEKKRARDPEMGGKQQRRRNPQEGVYNALQKDKMAEAYSEIGTKGERRRGKGHDGLYQGLSTATKDTYDALHMQTLA

SEQ ID NO: 11 - DNA, 66 bp, Artificial Sequence
  F2A nucleic acid sequence
gtgaaacagactttgaattttgaccttctgaagttggcaggagacgttgagtccaaccctgggccc

SEQ ID NO: 12 - protein, 22 aa, Artificial Sequence
  F2A amino acid sequence
VKQTLNFDLLKLAGDVESNPGP

SEQ ID NO: 13 - DNA, 462 bp, Artificial Sequence
  mouse IL7 nucleic acid sequence
atgttccatgtttcttttagatatatctttggaattcctccactgatccttgttctgctgcctgtcacatcatctgagtgccacattaaagacaaagaaggtaaagcatatgagagtgtactgatgatcagcatcgatgaattggacaaaatgacaggaactgatagtaattgcccgaataatgaaccaaacttttttagaaaacatgtatgtgatgatacaaaggaagctgcttttctaaatcgtgctgctcgcaagttgaagcaatttcttaaaatgaatatcagtgaagaattcaatgtccacttactaacagtatcacaaggcacacaaacactggtgaactgcacaagtaaggaagaaaaaaacgtaaaggaacagaaaaagaatgatgcatgtttcctaaagagactactgagagaaataaaaacttgttggaataaaattttgaagggcagtata

SEQ ID NO: 14 - DNA, 399 bp, Artificial Sequence
  mouse CCL21a nucleic acid sequence
atggctcagatgatgactctgagcctccttagcctggtcctggctctctgcatcccctggacccaaggcagtgatggagggggtcaggactgctgccttaagtacagccagaagaaaattccctacagtattgtccgaggctataggaagcaagaaccaagtttaggctgtcccatcccggcaatcctgttctcaccccggaagcactctaagcctgagctatgtgcaaaccctgaggaaggctgggtgcagaacctgatgcgccgcctggaccagcctccagccccagggaaacaaagccccggctgcaggaagaaccggggaacctctaagtctggaaagaaaggaaagggctccaagggctgcaagagaactgaacagacacagccctcaagagga

SEQ ID NO: 15 - DNA, 399 bp, Artificial Sequence
  mouse CCL21b nucleic acid sequence
atggctcagatgatgactctgagcctccttagcctggtcctggctctctgcatcccctggacccaaggcagtgatggagggggacaggactgctgccttaagtacagccagaagaaaattccctacagtattgtccgaggctataggaagcaagaaccaagtttaggctgtcccatcccggcaatcctgttcttaccccggaagcactctaagcctgagctatgtgcaaaccctgaggaaggctgggtgcagaacctgatgcgccgcctggaccagcctccagccccagggaaacaaagccccggctgcaggaagaaccggggaacctctaagtctggaaagaaaggaaagggctccaagggctgcaagagaactgaacagacacagccctcaagagga

SEQ ID NO: 16 - DNA, 57 bp, Artificial Sequence
  P2A nucleic acid sequence
gctactaacttcagcctgctgaagcaggctggagacgtggaggagaaccctggacct

SEQ ID NO: 17 - DNA, 534 bp, Artificial Sequence
  human IL7 nucleic acid sequence
atgttccatgtttcttttaggtatatctttggacttcctcccctgatccttgttctgttgccagtagcatcatctgattgtgatattgaaggtaaagatggcaaacaatatgagagtgttctaatggtcagcatcgatcaattattggacagcatgaaagaaattggtagcaattgcctgaataatgaatttaacttttttaaaagacatatctgtgatgctaataaggaaggtatgtttttattccgtgctgctcgcaagttgaggcaatttcttaaaatgaatagcactggtgattttgatctccacttattaaaagtttcagaaggcacaacaatactgttgaactgcactggccaggttaaaggaagaaaaccagctgccctgggtgaagcccaaccaacaaagagtttggaagaaaataaatctttaaaggaacagaaaaaactgaatgacttgtgtttcctaaagagactattacaagagataaaaacttgttggaataaaattttgatgggcactaaagaacactga

SEQ ID NO: 18 - protein, 177 aa, Artificial Sequence
  human IL7 amino acid sequence
MFHVSFRYIFGLPPLILVLLPVASSDCDIEGKDGKQYESVLMVSIDQLLDSMKEIGSNCLNNEFNFFKRHICDANKEGMFLFRAARKLRQFLKMNSTGDFDLHLLKVSEGTTILLNCTGQVKGRKPAALGEAQPTKSLEENKSLKEQKKLNDLCFLKRLLQEIKTCWNKILMGTKEH

SEQ ID NO: 19 - protein, 459 aa, Artificial Sequence
  human IL7R amino acid sequence
MTILGTTFGMVFSLLQVVSGESGYAQNGDLEDAELDDYSFSCYSQLEVNGSQHSLTCAFEDPDVNITNLEFEICGALVEVKCLNFRKLQEIYFIETKKFLLIGKSNICVKVGEKSLTCKKIDLTTIVKPEAPFDLSVVYREGANDFVVTFNTSHLQKKYVKVLMHDVAYRQEKDENKWTHVNLSSTKLTLLQRKLQPAAMYEIKVRSIPDHYFKGFWSEWSPSYYFRTPEINNSSGEMDPILLTISILSFFSVALLVILACVLWKKRIKPIVWPSLPDHKKTLEHLCKKPRKNLNVSFNPESFLDCQIHRVDDIQARDEVEGFLQDTFPQQLEESEKQRLGGDVQSPNCPSEDVVITPESFGRDSSLTCLAGNVSACDAPILSSSRSLDCRESGKNGPHVYQDLLLSLGTTNSTLPPPFSLQSGILTLNPVAQGQPILTSLGSNQEEAYVTMSSFYQNQ

SEQ ID NO: 20 - DNA, 405 bp, Artificial Sequence
  human CCL21 nucleic acid sequence
atggctcagtcactggctctgagcctccttatcctggttctggcctttggcatccccaggacccaaggcagtgatggaggggctcaggactgttgcctcaagtacagccaaaggaagattcccgccaaggttgtccgcagctaccggaagcaggaaccaagcttaggctgctccatcccagctatcctgttcttgccccgcaagcgctctcaggcagagctatgtgcagacccaaaggagctctgggtgcagcagctgatgcagcatctggacaagacaccatccccacagaaaccagcccagggctgcaggaaggacaggggggcctccaagactggcaagaaaggaaagggctccaaaggctgcaagaggactgagcggtcacagacccctaaagggccatag

SEQ ID NO: 21 - protein, 134 aa, Artificial Sequence
  human CCL21 amino acid sequence
MAQSLALSLLILVLAFGIPRTQGSDGGAQDCCLKYSQRKIPAKVVRSYRKQEPSLGCSIPAILFLPRKRSQAELCADPKELWVQQLMQHLDKTPSPQKPAQGCRKDRGASKTGKKGKGSKGCKRTERSQTPKGP

SEQ ID NO: 22 - protein, 261 aa, Artificial Sequence
  Claudin18.2 amino acid sequence
MAVTACQGLGFVVSLIGIAGIIAATCMDQWSTQDLYNNPVTAVFNYQGLWRSCVRESSGFTECRGYFTLLGLPAMLQAVRALMIVGIVLGAIGLLVSIFALKCIRIGSMEDSAKANMTLTSGIMFIVSGLCAIAGVSVFANMLVTNFWMSTANMYTGMGGMVQTVQTRYTFGAALFVGWVAGGLTLIGGVMMCIACRGLAPEETNYKAVSYHASGHSVAYKPGGFKASTGFGSNTKNKKIYDGGARTEDEVQSYPSKHDYV

SEQ ID NO: 23 - protein, 261 aa, Artificial Sequence
  Claudin18.1 amino acid sequence
MSTTTCQVVAFLLSILGLAGCIAATGMDMWSTQDLYDNPVTSVFQYEGLWRSCVRQSSGFTECRPYFTILGLPAMLQAVRALMIVGIVLGAIGLLVSIFALKCIRIGSMEDSAKANMTLTSGIMFIVSGLCAIAGVSVFANMLVTNFWMSTANMYTGMGGMVQTVQTRYTFGAALFVGWVAGGLTLIGGVMMCIACRGLAPEETNYKAVSYHASGHSVAYKPGGFKASTGFGSNTKNKKIYDGGARTEDEVQSYPSKHDYV

SEQ ID NO: 24 - DNA, 135 bp, Artificial Sequence
  mouse4-1BB intracellular domain nucleic acid sequence
aaatggatcaggaaaaaattcccccacatattcaagcaaccatttaagaagaccactggagcagctcaagaggaagatgcttgtagctgccgatgtccacaggaagaagaaggaggaggaggaggctatgagctg

SEQ ID NO: 25 - protein, 45 aa, Artificial Sequence
  mouse4-1BB intracellular domain amino acid sequence
KWIRKKFPHIFKQPFKKTTGAAQEEDACSCRCPQEEEGGGGGYEL

SEQ ID NO: 26 - protein, 473 aa, Artificial Sequence
  Hu8E5-28ZCAR amino acid sequence (human)
QVQLQESGPGLIKPSQTLSLTCTVSGGSISSGYNWHWIRQPPGKGLEWIGYIHYTGSTNYNPALRSRVTISVDTSKNQFSLKLSSVTAADTAIYYCARIYNGNSFPYWGQGTTVTVSSGGGGSGGGGSGGGGSDIVMTQSPDSLAVSLGERATINCKSSQSLFNSGNQKNYLTWYQQKPGQPPKLLIYWASTRESGVPDRFSGSGSGTDFTLTISSLQAEDVAVYYCQNAYSFPYTFGGGTKLEIKRTTTPAPRPPTPAPTIASQPLSLRPEACRPAAGGAVHTRGLDFACDFWVLVVVGGVLACYSLLVTVAFIIFWVRSKRSRLLHSDYMNMTPRRPGPTRKHYQPYAPPRDFAAYRSRVKFSRSADAPAYQQGQNQLYNELNLGRREEYDVLDKRRGRDPEMGGKPQRRKNPQEGLYNELQKDKMAEAYSEIGMKGERRRGKGHDGLYQGLSTATKDTYDALHMQALPPR

SEQ ID NO: 27 - protein, 471 aa, Artificial Sequence
  Hu8E5-BBZCAR amino acid sequence (human)
QVQLQESGPGLIKPSQTLSLTCTVSGGSISSGYNWHWIRQPPGKGLEWIGYIHYTGSTNYNPALRSRVTISVDTSKNQFSLKLSSVTAADTAIYYCARIYNGNSFPYWGQGTTVTVSSGGGGSGGGGSGGGGSDIVMTQSPDSLAVSLGERATINCKSSQSLFNSGNQKNYLTWYQQKPGQPPKLLIYWASTRESGVPDRFSGSGSGTDFTLTISSLQAEDVAVYYCQNAYSFPYTFGGGTKLEIKRTTTPAPRPPTPAPTIASQPLSLRPEACRPAAGGAVHTRGLDFACDIYIWAPLAGTCGVLLLSLVITLYCKRGRKKLLYIFKQPFMRPVQTTQEEDGCSCRFPEEEEGGCELRVKFSRSADAPAYQQGQNQLYNELNLGRREEYDVLDKRRGRDPEMGGKPQRRKNPQEGLYNELQKDKMAEAYSEIGMKGERRRGKGHDGLYQGLSTATKDTYDALHMQALPPR

SEQ ID NO: 28 - protein, 21 aa, Artificial Sequence
  human CD8 alpha signal peptide amino acid sequence
MALPVTALLLPLALLLHAARP

SEQ ID NO: 29 - protein, 45 aa, Artificial Sequence
  humanCD8 hinge region amino acid sequence
TTTPAPRPPTPAPTIASQPLSLRPEACRPAAGGAVHTRGLDFACD

SEQ ID NO: 30 - protein, 27 aa, Artificial Sequence
  human CD28 Transmembrane amino acid sequence
FWVLVVVGGVLACYSLLVTVAFIIFWV

SEQ ID NO: 31 - protein, 41 aa, Artificial Sequence
  human CD28 intracellular domain amino acid sequence
RSKRSRLLHSDYMNMTPRRPGPTRKHYQPYAPPRDFAAYRS

SEQ ID NO: 32 - protein, 42 aa, Artificial Sequence
  human 4-1BB intracellular domain amino acid sequence
KRGRKKLLYIFKQPFMRPVQTTQEEDGCSCRFPEEEEGGCEL

SEQ ID NO: 33 - protein, 113 aa, Artificial Sequence
  intracellular segment CD3 xi amino acid sequence of human CD3
RVKFSRSADAPAYQQGQNQLYNELNLGRREEYDVLDKRRGRDPEMGGKPQRRKNPQEGLYNELQKDKMAEAYSEIGMKGERRRGKGHDGLYQGLSTATKDTYDALHMQALPPR

SEQ ID NO: 34 - DNA, 324 bp, Artificial Sequence
  mouse CCL19 nucleic acid sequence
atggccccccgtgtgaccccactcctggccttcagcctgctggttctctggaccttcccagccccaactctggggggtgctaatgatgcggaagactgctgcctgtctgtgacccagcgccccatccctgggaacatcgtgaaagccttccgctaccttcttaatgaagatggctgcagggtgcctgctgttgtgttcaccacactaaggggctatcagctctgtgcacctccagaccagccctgggtggatcgcatcatccgaagactgaagaagtcttctgccaagaacaaaggcaacagcaccagaaggagccctgtgtct

SEQ ID NO: 35 - protein, 515 aa, Artificial Sequence
  28BBZ amino acid sequence
QVQLQESGPGLIKPSQTLSLTCTVSGGSISSGYNWHWIRQPPGKGLEWIGYIHYTGSTNYNPALRSRVTISVDTSKNQFSLKLSSVTAADTAIYYCARIYNGNSFPYWGQGTTVTVSSGGGGSGGGGSGGGGSDIVMTQSPDSLAVSLGERATINCKSSQSLFNSGNQKNYLTWYQQKPGQPPKLLIYWASTRESGVPDRFSGSGSGTDFTLTISSLQAEDVAVYYCQNAYSFPYTFGGGTKLEIKRTTTPAPRPPTPAPTIASQPLSLRPEACRPAAGGAVHTRGLDFACDFWVLVVVGGVLACYSLLVTVAFIIFWVRSKRSRLLHSDYMNMTPRRPGPTRKHYQPYAPPRDFAAYRSKRGRKKLLYIFKQPFMRPVQTTQEEDGCSCRFPEEEEGGCELRVKFSRSADAPAYQQGQNQLYNELNLGRREEYDVLDKRRGRDPEMGGKPQRRKNPQEGLYNELQKDKMAEAYSEIGMKGERRRGKGHDGLYQGLSTATKDTYDALHMQALPPR